European Patent Specification EP 3 466 427 B1, published July 22, 2026. Title: Sleep-improving agent. Applicant: AMINO UP CHEMICAL CO., LTD. OTSUKA PHARMACEUTICAL CO., LTD. The sequence listing filed with the application follows.

SEQUENCE LISTING (4 sequences)

SEQ ID NO: 1 - DNA, 24 bp, HSP70 forward primer
gcatttcctagtatttctgtttgt

SEQ ID NO: 2 - DNA, 23 bp, HSP70 reverse primer
aatagtcgtaagatggcagtata

SEQ ID NO: 3 - DNA, 19 bp, beta 2 microglobulin forward primer
tagctgtgctcgcgctact

SEQ ID NO: 4 - DNA, 20 bp, beta 2 microglobulin reverse primer
agtgggggtgaattcagtgt